European Patent Specification EP 4 453 236 B1, published September 10, 2025. Title: METHODS AND SYSTEMS FOR ANALYZING TARGET ENGAGEMENT DATA FROM BIOLOGICAL ASSAYS. Applicant: THE UNITED STATES OF AMERICA, AS REPRESENTED BY THE SECRETARY, DEPARTMENT OF HEALTH AND HUMAN SERVICES. The sequence listing filed with the application follows.

SEQUENCE LISTING (29 sequences)

SEQ ID NO: 1 - protein, 7 aa, synthetic construct
  REGION 1..7: note = Synthetic
GSGGGGS

SEQ ID NO: 2 - protein, 17 aa, synthetic construct
  REGION 1..17: note = Synthetic
GSGGGGSGGGGSGGGGS

SEQ ID NO: 3 - protein, 12 aa, synthetic construct
  REGION 1..12: note = Synthetic
AEAAAKEAAAKA

SEQ ID NO: 4 - protein, 46 aa, synthetic construct
  REGION 1..46: note = Synthetic
AEAAAKEAAAKEAAAKEAAAKALEAEAAAKEAAAKEAAAKEAAAKA

SEQ ID NO: 5 - protein, 32 aa, synthetic construct
  REGION 1..32: note = Synthetic
AEAAAKEAAAKEAAAKEAAAKEAAAKEAAAKA

SEQ ID NO: 6 - protein, 7 aa, synthetic construct
  REGION 1..7: note = Synthetic
AEAAAKA

SEQ ID NO: 7 - protein, 17 aa, synthetic construct
  REGION 1..17: note = Synthetic
AEAAAKEAAAKEAAAKA

SEQ ID NO: 8 - protein, 22 aa, synthetic construct
  REGION 1..22: note = Synthetic
AEAAAKEAAAKEAAAKEAAAKA

SEQ ID NO: 9 - protein, 27 aa, synthetic construct
  REGION 1..27: note = Synthetic
AEAAAKEAAAKEAAAKEAAAKEAAAKA

SEQ ID NO: 10 - protein, 10 aa, synthetic construct
  REGION 1..10: note = Synthetic
APAPAPAPAP

SEQ ID NO: 11 - protein, 20 aa, synthetic construct
  REGION 1..20: note = Synthetic
APAPAPAPAPAPAPAPAPAP

SEQ ID NO: 12 - protein, 30 aa, synthetic construct
  REGION 1..30: note = Synthetic
APAPAPAPAPAPAPAPAPAPAPAPAPAPAP

SEQ ID NO: 13 - protein, 40 aa, synthetic construct
  REGION 1..40: note = Synthetic
APAPAPAPAPAPAPAPAPAPAPAPAPAPAPAPAPAPAPAP

SEQ ID NO: 14 - protein, 20 aa, synthetic construct
  REGION 1..20: note = Synthetic
PPPPPPPPPPPPPPPPPPPP

SEQ ID NO: 15 - protein, 30 aa, synthetic construct
  REGION 1..30: note = Synthetic
PPPPPPPPPPPPPPPPPPPPPPPPPPPPPP

SEQ ID NO: 16 - protein, 20 aa, synthetic construct
  REGION 1..20: note = Synthetic
SSSSSSSSSSSSSSSSSSSS

SEQ ID NO: 17 - protein, 40 aa, synthetic construct
  REGION 1..40: note = Synthetic
SSSSSSSSSSSSSSSSSSSSSSSSSSSSSSSSSSSSSSSS

SEQ ID NO: 18 - protein, 159 aa, synthetic construct
  REGION 1..159: note = Synthetic
MVFTLEDFVGDWEQTAAYNLDQVLEQGGVSSLLQNLAVSVTPIQRIVRSGENALKIDIHVIIPYEGLSADQMAQIEEVFKVVYPVDDHHFKVILPYGTLVIDGVTPNMLNYFGRPYEGIAVFDGKKITVTGTLWNGNKIIDERLITPDGSMLFRVTINS

SEQ ID NO: 19 - protein, 12 aa, synthetic construct
  REGION 1..12: note = Synthetic
GSGSGSGSGSGS

SEQ ID NO: 20 - protein, 11 aa, synthetic construct
  REGION 1..11: note = Synthetic
VSGWRLFKKIS

SEQ ID NO: 21 - protein, 13 aa, synthetic construct
  REGION 1..13: note = Synthetic
VSGWRLFKKISGS

SEQ ID NO: 22 - protein, 15 aa, synthetic construct
  REGION 1..15: note = Synthetic
GSVSGWRLFKKISGS

SEQ ID NO: 23 - protein, 184 aa, synthetic construct
  REGION 1..184: note = Synthetic
MVFTLEDFVGDWEQTAAYNLDQVLEQGGVSSLLQNLAVSVTPIQRIVRSGENALKIDIHVIIPYEGLSADQMAQIEEVFKVVYPVDDHHFKVILPYGTLVIDGVTPNMLNYFGRPYEGIAVFDGKKITVTGTLWNGNKIIDERLITPDGSMLFRVTINSGSGSGSGSGSGSVSGWRLFKKISGS

SEQ ID NO: 24 - DNA, 477 bp, synthetic construct
  misc_feature 1..477: note = Synthetic
  source 1..477: mol_type = other DNA
atggtcttcacactcgaagatttcgttggggactgggaacagacagccgcctacaacctggaccaagtccttgaacagggaggtgtgtccagtttgctgcagaatctcgccgtgtccgtaactccgatccaaaggattgtccggagcggtgaaaatgccctgaagatcgacatccatgtcatcatcccgtatgaaggtctgagcgccgaccaaatggcccagatcgaagaggtgtttaaggtggtgtaccctgtggatgatcatcactttaaggtgatcctgccctatggcacactggtaatcgacggggttacgccgaacatgctgaactatttcggacggccgtatgaaggcatcgccgtgttcgacggcaaaaagatcactgtaacagggaccctgtggaacggcaacaaaattatcgacgagcgcctgatcacccccgacggctccatgctgttccgagtaaccatcaacagt

SEQ ID NO: 25 - DNA, 33 bp, synthetic construct
  misc_feature 1..33: note = Synthetic
  source 1..33: mol_type = other DNA
gtgagtggctggcgactgttcaagaagatcagc

SEQ ID NO: 26 - DNA, 39 bp, synthetic construct
  misc_feature 1..39: note = Synthetic
  source 1..39: mol_type = other DNA
gtgagtggctggcgactgttcaagaagatcagcggcagc

SEQ ID NO: 27 - DNA, 45 bp, synthetic construct
  misc_feature 1..45: note = Synthetic
  source 1..45: mol_type = other DNA
ggatccgtgagtggctggcgactgttcaagaagatcagcggcagc

SEQ ID NO: 28 - DNA, 555 bp, synthetic construct
  misc_feature 1..555: note = Synthetic
  source 1..555: mol_type = other DNA
atggtcttcacactcgaagatttcgttggggactgggaacagacagccgcctacaacctggaccaagtccttgaacagggaggtgtgtccagtttgctgcagaatctcgccgtgtccgtaactccgatccaaaggattgtccggagcggtgaaaatgccctgaagatcgacatccatgtcatcatcccgtatgaaggtctgagcgccgaccaaatggcccagatcgaagaggtgtttaaggtggtgtaccctgtggatgatcatcactttaaggtgatcctgccctatggcacactggtaatcgacggggttacgccgaacatgctgaactatttcggacggccgtatgaaggcatcgccgtgttcgacggcaaaaagatcactgtaacagggaccctgtggaacggcaacaaaattatcgacgagcgcctgatcacccccgacggctccatgctgttccgagtaaccatcaacagtggtagcggtagcggtagcggtagcggtagcggatccgtgagtggctggcgactgttcaagaagatcagcggcagctaa

SEQ ID NO: 29 - DNA, 36 bp, synthetic construct
  misc_feature 1..36: note = Synthetic
  source 1..36: mol_type = other DNA
ggtagcggtagcggtagcggtagcggtagcggatcc